European Patent Application EP 4 253 413 A1, published October 4, 2023. Title: HUMAN LIFR ANTIGEN BINDING PROTEIN, PREPARATION METHOD THEREFOR, AND APPLICATION THEREOF. Applicant: Nona Biosciences (Suzhou) Co., Ltd. Yinuoke Biomedical Co., Ltd. Application 21914475.5. The sequence listing filed with the application follows.

SEQUENCE LISTING (103 sequences)

SEQ ID NO: 1 - protein, 10 aa, artificial sequence
GFTFSSYGMH

SEQ ID NO: 2 - protein, 10 aa, artificial sequence
GFTFSSYGMD

SEQ ID NO: 3 - protein, 10 aa, artificial sequence
GFTFSSYGMN

SEQ ID NO: 4 - protein, 10 aa, artificial sequence
GFTFSNYAMT

SEQ ID NO: 5 - protein, 17 aa, artificial sequence
VIWYDGNNKYYADSVKG

SEQ ID NO: 6 - protein, 17 aa, artificial sequence
VIWYDGSNKYYEDSVKG

SEQ ID NO: 7 - protein, 17 aa, artificial sequence
VIWYDGSNKFYADSVRG

SEQ ID NO: 8 - protein, 17 aa, artificial sequence
VIWYDGSNKYYADSVKG

SEQ ID NO: 9 - protein, 17 aa, artificial sequence
VIWYDGSNKYYTDSVKG

SEQ ID NO: 10 - protein, 17 aa, artificial sequence
VIWFDGSNKYYADSVKG

SEQ ID NO: 11 - protein, 17 aa, artificial sequence
VIWFDGSIKYYADSVKG

SEQ ID NO: 12 - protein, 17 aa, artificial sequence
VIWFDGSLKYYADSVKG

SEQ ID NO: 13 - protein, 17 aa, artificial sequence
VIWFDGSVKYYADSVKG

SEQ ID NO: 14 - protein, 17 aa, artificial sequence
TISGSGAFTYYADAVKG

SEQ ID NO: 15 - protein, 17 aa, artificial sequence
VISGSGFLTYYADAVKG

SEQ ID NO: 16 - protein, 16 aa, artificial sequence
DGESSMVRGLLNWFDP

SEQ ID NO: 17 - protein, 14 aa, artificial sequence
ELRYFDWLLSPFDY

SEQ ID NO: 18 - protein, 13 aa, artificial sequence
ELWFGELLSPLDF

SEQ ID NO: 19 - protein, 13 aa, artificial sequence
ELWFGELLSPFDF

SEQ ID NO: 20 - protein, 7 aa, artificial sequence
GQLVGDY

SEQ ID NO: 21 - protein, 7 aa, artificial sequence
GERTLDL

SEQ ID NO: 22 - protein, 7 aa, artificial sequence
GQLVQDF

SEQ ID NO: 23 - protein, 7 aa, artificial sequence
GQLVQDL

SEQ ID NO: 24 - protein, 9 aa, artificial sequence
GGILTGFDN

SEQ ID NO: 25 - protein, 9 aa, artificial sequence
GGILTGFDY

SEQ ID NO: 26 - protein, 12 aa, artificial sequence
RASQSVSSSYLA

SEQ ID NO: 27 - protein, 12 aa, artificial sequence
RASQSVSSSFLA

SEQ ID NO: 28 - protein, 12 aa, artificial sequence
RASQSISSSYLA

SEQ ID NO: 29 - protein, 11 aa, artificial sequence
RASQSISSYLN

SEQ ID NO: 30 - protein, 11 aa, artificial sequence
RASQSISSWLA

SEQ ID NO: 31 - protein, 11 aa, artificial sequence
RASQSISSNLA

SEQ ID NO: 32 - protein, 11 aa, artificial sequence
RASQNLNSNLA

SEQ ID NO: 33 - protein, 7 aa, artificial sequence
GASSRAT

SEQ ID NO: 34 - protein, 7 aa, artificial sequence
GTSSRAT

SEQ ID NO: 35 - protein, 7 aa, artificial sequence
AASNRAT

SEQ ID NO: 36 - protein, 7 aa, artificial sequence
AASSLQS

SEQ ID NO: 37 - protein, 7 aa, artificial sequence
KASSLES

SEQ ID NO: 38 - protein, 7 aa, artificial sequence
KASNLES

SEQ ID NO: 39 - protein, 7 aa, artificial sequence
KASNLEN

SEQ ID NO: 40 - protein, 7 aa, artificial sequence
GASTRAP

SEQ ID NO: 41 - protein, 9 aa, artificial sequence
QQYGSSPFT

SEQ ID NO: 42 - protein, 9 aa, artificial sequence
QQSYSTPLT

SEQ ID NO: 43 - protein, 12 aa, artificial sequence
QQYKSFSPGGLT

SEQ ID NO: 44 - protein, 9 aa, artificial sequence
QQYKSNPLT

SEQ ID NO: 45 - protein, 9 aa, artificial sequence
QQYNNWPRT

SEQ ID NO: 46 - protein, 125 aa, artificial sequence
QVQLVESGGGVVQPGRSLRLSCAASGFTFSSYGMHWVRQAPGKGLEWVAVIWYDGNNKYYADSVKGRFTISRDNSKNTLYLQMNSLRAEDTAVYYCARDGESSMVRGLLNWFDPWGQGTLVTVSS

SEQ ID NO: 47 - protein, 122 aa, artificial sequence
QVQLVESGGGVVQPGRSLRLSCAASGFTFSSYGMDWVRQAPGKGLEWVAVIWYDGSNKYYADSVKGRFTISRDNSKNTLYLQMNSLRAEDTAVYYCARELWFGELLSPFDFWGQGTLVTVSS

SEQ ID NO: 48 - protein, 116 aa, artificial sequence
QGQLVESGGGVVQPGRSLRLSCAASGFTFSSYGMHWVRQPPGKGLEWVAVIWFDGSNKYYADSVKGRFTISRDNSKNTVYLQMDSLRDEDTAVYYCARGQLVGDYWGQGTLVTVSS

SEQ ID NO: 49 - protein, 122 aa, artificial sequence
QVQLVESGGGVVQPGKSLRLSCAASGFTFSSYGMDWVRQAPGKGLEWVAVIWYDGSNKYYTDSVKGRFTISRDNSKNTLYLQMNSLRAEDTAVYYCARELWFGELLSPFDFWGQGTLVTVSS

SEQ ID NO: 50 - protein, 123 aa, artificial sequence
QVQLVESGGGVVQPGRSLRLSCAASGFTFSSYGMHWVRQAPGKGLEWVAVIWYDGSNKYYEDSVKGRFTISRDNSKNTLYLQMNSLRAEDTAVYYCARELRYFDWLLSPFDYWGQGTLVTVSS

SEQ ID NO: 51 - protein, 122 aa, artificial sequence
QVQLVESGGGVVQPGRSLRLSCAASGFTFSSYGMDWVRQAPGKGLEWVAVIWYDGSNKFYADSVRGRFTISRDNSQNTLYLQMNSLRAEDTAVYYCARELWFGELLSPLDFWGQGTLVTVSS

SEQ ID NO: 52 - protein, 122 aa, artificial sequence
QVQLVESGGGVVQPGRSLRLSCAASGFTFSSYGMDWVRQAPGKGLEWVAVIWYDGSNKFYADSVRGRFTISRDNSQNTLYLQMNSLRAEDTAVYYCARELWFGELLSPFDFWGQGTLVTVSS

SEQ ID NO: 53 - protein, 116 aa, artificial sequence
QVQLVESGGGVVQPGRSLRLSCVASGFTFSSYGMNWVRQAPGKGLDWVTVIWFDGSNKYYADSVKGRFTISRDNSKNTLYLQMNSLRAEDTAMYYCARGERTLDLWGQGTLVTVSS

SEQ ID NO: 54 - protein, 116 aa, artificial sequence
QVQLVESGGGVVQPGRSLRLSCAASGFTFSSYGMNWVRQAPGKGLEWVAVIWFDGSIKYYADSVKGRFTISRDNSKNTLYLQMNSLRAEDTAIYYCARGQLVQDFWGRGTLVTVSS

SEQ ID NO: 55 - protein, 116 aa, artificial sequence
QVQLVESGGGVVQPGRSLRLSCAASGFTFSSYGMHWVRQAPGKGLEWVAVIWFDGSLKYYADSVKGRFAISRDNSKNTLYLQMNSLRAEDTAIFYCARGQLVQDLWGRGTLVTVSS

SEQ ID NO: 56 - protein, 116 aa, artificial sequence
QVQLVESGGGVVQPGRSLRLSCAASGFTFSSYGMHWVRQAPGKGLEWVAVIWFDGSIKYYADSVKGRFTISRDNSKNTLYLQMNSLRAEDTAIYYCARGQLVQDFWGRGTLVTVSS

SEQ ID NO: 57 - protein, 116 aa, artificial sequence
QVQLVESGGGVVQPGRSLRLSCAASGFTFSSYGMHWVRQAPGKGLEWVAVIWFDGSVKYYADSVKGRFTISRDNSKNTLYLQMNSLRAEDTAIYYCARGQLVQDFWGRGTLVTVSS

SEQ ID NO: 58 - protein, 118 aa, artificial sequence
EVQLLQSGGGLVQPGGSLRLSCAASGFTFSNYAMTWVRQAPGKGLEWVSTISGSGAFTYYADAVKGRFTISRVNSKNSLDLQMNSLRAEDTAVYYCAKGGILTGFDNWGQGTLVTVSS

SEQ ID NO: 59 - protein, 117 aa, artificial sequence
EVQLLESGGGLVQPGGSLRLSCATSGFTFSNYAMTWVRQAPGKGLEWVVISGSGFLTYYADAVKGRFTISRVNSKNSLYLQMNSLRAEDTAVYYCTKGGILTGFDYWGQGTLVTVSS

SEQ ID NO: 60 - protein, 108 aa, artificial sequence
EIVLTQSPGTLSLSPGERATLSCRASQSVSSSYLAWYQQKPGQAPRLLIYGASSRATGIPDRFSGSGSGTDFTLTISRLEPEDFAVYYCQQYGSSPFTFGPGTKVDIK

SEQ ID NO: 61 - protein, 108 aa, artificial sequence
KIVLTQSPGTLSLSPGGRATLSCRASQSISSSYLAWYQQKPGQAPRLLIYAASNRATGIPDRFSGSGSGTDFTLTISRLEPEDFAVYYCQQYGSSPFTFGPGIKVDIK

SEQ ID NO: 62 - protein, 107 aa, artificial sequence [sequence omitted]

SEQ ID NO: 63 - protein, 108 aa, artificial sequence
EIVLTQSPGPLSLSPGERATLSCRASQSVSSSFLAWYQQKPGQAPRLLIYGTSSRATGIPDRFSGSGSGTDFTLTISRLEPEDFAVYYCQQYGSSPFTFGPGTKVGIK

SEQ ID NO: 64 - protein, 108 aa, artificial sequence
EIVLTQSPGTLSLSPGGRATLSCRASQSVSSSYLAWYQQKPGQAPRLLIYGASSRATGIPDRFSGSGSGTDFTLTISRLEPEDFAVYYCQQYGSSPFTFGPGIKVDIK

SEQ ID NO: 65 - protein, 108 aa, artificial sequence; identical to SEQ ID NO: 64

SEQ ID NO: 66 - protein, 110 aa, artificial sequence
DIQMTQSPSTLSASVGDRVTITCRASQSISSWLAWYQQKPGKAPKLLIYKASSLESGVPSRFSGSGSGTEFSFTISSLQPDDFATYYCQQYKSFSPGGLTFGGGTKVEIK

SEQ ID NO: 67 - protein, 107 aa, artificial sequence
DIQMTQSPSTLSASVGDRVTITCRASQSISSWLAWYQQKPGKAPNLLMYKASNLESGVPSRFSGSGSGTEFTLTITSLQPDDFASYYCQQYKSNPLTFGGGTKVEIK

SEQ ID NO: 68 - protein, 107 aa, artificial sequence
DIQMTQSPSTLSASVGDRVTITCRASQSISSWLAWYQQKPGKAPNLLMYKASNLENGVSSRFSGSGSGTEFTLTITSLQPDDFATYYCQQYKSNPLTFGGGTKVEIK

SEQ ID NO: 69 - protein, 107 aa, artificial sequence
KIVMTQSPATLSVSPGERATLSCRASQNLNSNLAWYQQTPGQAPRLLIYGASTRAPGIPARFSGSGSGTEFTLTISSLQSEDFVVYFCQQYNNWPRTFGQGTKVEIK

SEQ ID NO: 70 - protein, 453 aa, artificial sequence
QVQLVESGGGVVQPGRSLRLSCAASGFTFSSYGMHWVRQAPGKGLEWVAVIWYDGNNKYYADSVKGRFTISRDNSKNTLYLQMNSLRAEDTAVYYCARDGESSMVRGLLNWFDPWGQGTLVTVSSASTKGPSVFPLAPSSKSTSGGTAALGCLVKDYFPEPVTVSWNSGALTSGVHTFPAVLQSSGLYSLSSVVTVPSSSLGTQTYICNVNHKPSNTKVDKKVEPKSCDKTHTCPPCPAPELLGGPSVFLFPPKPKDTLMISRTPEVTCVVVDVSHEDPEVKFNWYVDGVEVHNAKTKPREEQYNSTYRVVSVLTVLHQDWLNGKEYKCKVSNKALPAPIEKTISKAKGQPREPQVYTLPPSREEMTKNQVSLTCLVKGFYPSDIAVEWESNGQPENNYKTTPPVLDSDGSFFLYSKLTVDKSRWQQGNVFSCSVMHEALHNHYTQKSLSLSP

SEQ ID NO: 71 - protein, 450 aa, artificial sequence
QVQLVESGGGVVQPGRSLRLSCAASGFTFSSYGMDWVRQAPGKGLEWVAVIWYDGSNKYYADSVKGRFTISRDNSKNTLYLQMNSLRAEDTAVYYCARELWFGELLSPFDFWGQGTLVTVSSASTKGPSVFPLAPSSKSTSGGTAALGCLVKDYFPEPVTVSWNSGALTSGVHTFPAVLQSSGLYSLSSVVTVPSSSLGTQTYICNVNHKPSNTKVDKKVEPKSCDKTHTCPPCPAPELLGGPSVFLFPPKPKDTLMISRTPEVTCVVVDVSHEDPEVKFNWYVDGVEVHNAKTKPREEQYNSTYRVVSVLTVLHQDWLNGKEYKCKVSNKALPAPIEKTISKAKGQPREPQVYTLPPSREEMTKNQVSLTCLVKGFYPSDIAVEWESNGQPENNYKTTPPVLDSDGSFFLYSKLTVDKSRWQQGNVFSCSVMHEALHNHYTQKSLSLSP

SEQ ID NO: 72 - protein, 444 aa, artificial sequence
QGQLVESGGGVVQPGRSLRLSCAASGFTFSSYGMHWVRQPPGKGLEWVAVIWFDGSNKYYADSVKGRFTISRDNSKNTVYLQMDSLRDEDTAVYYCARGQLVGDYWGQGTLVTVSSASTKGPSVFPLAPSSKSTSGGTAALGCLVKDYFPEPVTVSWNSGALTSGVHTFPAVLQSSGLYSLSSVVTVPSSSLGTQTYICNVNHKPSNTKVDKKVEPKSCDKTHTCPPCPAPELLGGPSVFLFPPKPKDTLMISRTPEVTCVVVDVSHEDPEVKFNWYVDGVEVHNAKTKPREEQYNSTYRVVSVLTVLHQDWLNGKEYKCKVSNKALPAPIEKTISKAKGQPREPQVYTLPPSREEMTKNQVSLTCLVKGFYPSDIAVEWESNGQPENNYKTTPPVLDSDGSFFLYSKLTVDKSRWQQGNVFSCSVMHEALHNHYTQKSLSLSP

SEQ ID NO: 73 - protein, 450 aa, artificial sequence
QVQLVESGGGVVQPGKSLRLSCAASGFTFSSYGMDWVRQAPGKGLEWVAVIWYDGSNKYYTDSVKGRFTISRDNSKNTLYLQMNSLRAEDTAVYYCARELWFGELLSPFDFWGQGTLVTVSSASTKGPSVFPLAPSSKSTSGGTAALGCLVKDYFPEPVTVSWNSGALTSGVHTFPAVLQSSGLYSLSSVVTVPSSSLGTQTYICNVNHKPSNTKVDKKVEPKSCDKTHTCPPCPAPELLGGPSVFLFPPKPKDTLMISRTPEVTCVVVDVSHEDPEVKFNWYVDGVEVHNAKTKPREEQYNSTYRVVSVLTVLHQDWLNGKEYKCKVSNKALPAPIEKTISKAKGQPREPQVYTLPPSREEMTKNQVSLTCLVKGFYPSDIAVEWESNGQPENNYKTTPPVLDSDGSFFLYSKLTVDKSRWQQGNVFSCSVMHEALHNHYTQKSLSLSP

SEQ ID NO: 74 - protein, 451 aa, artificial sequence
QVQLVESGGGVVQPGRSLRLSCAASGFTFSSYGMHWVRQAPGKGLEWVAVIWYDGSNKYYEDSVKGRFTISRDNSKNTLYLQMNSLRAEDTAVYYCARELRYFDWLLSPFDYWGQGTLVTVSSASTKGPSVFPLAPSSKSTSGGTAALGCLVKDYFPEPVTVSWNSGALTSGVHTFPAVLQSSGLYSLSSVVTVPSSSLGTQTYICNVNHKPSNTKVDKKVEPKSCDKTHTCPPCPAPELLGGPSVFLFPPKPKDTLMISRTPEVTCVVVDVSHEDPEVKFNWYVDGVEVHNAKTKPREEQYNSTYRVVSVLTVLHQDWLNGKEYKCKVSNKALPAPIEKTISKAKGQPREPQVYTLPPSREEMTKNQVSLTCLVKGFYPSDIAVEWESNGQPENNYKTTPPVLDSDGSFFLYSKLTVDKSRWQQGNVFSCSVMHEALHNHYTQKSLSLSP

SEQ ID NO: 75 - protein, 450 aa, artificial sequence
QVQLVESGGGVVQPGRSLRLSCAASGFTFSSYGMDWVRQAPGKGLEWVAVIWYDGSNKFYADSVRGRFTISRDNSQNTLYLQMNSLRAEDTAVYYCARELWFGELLSPLDFWGQGTLVTVSSASTKGPSVFPLAPSSKSTSGGTAALGCLVKDYFPEPVTVSWNSGALTSGVHTFPAVLQSSGLYSLSSVVTVPSSSLGTQTYICNVNHKPSNTKVDKKVEPKSCDKTHTCPPCPAPELLGGPSVFLFPPKPKDTLMISRTPEVTCVVVDVSHEDPEVKFNWYVDGVEVHNAKTKPREEQYNSTYRVVSVLTVLHQDWLNGKEYKCKVSNKALPAPIEKTISKAKGQPREPQVYTLPPSREEMTKNQVSLTCLVKGFYPSDIAVEWESNGQPENNYKTTPPVLDSDGSFFLYSKLTVDKSRWQQGNVFSCSVMHEALHNHYTQKSLSLSP

SEQ ID NO: 76 - protein, 450 aa, artificial sequence
QVQLVESGGGVVQPGRSLRLSCAASGFTFSSYGMDWVRQAPGKGLEWVAVIWYDGSNKFYADSVRGRFTISRDNSQNTLYLQMNSLRAEDTAVYYCARELWFGELLSPFDFWGQGTLVTVSSASTKGPSVFPLAPSSKSTSGGTAALGCLVKDYFPEPVTVSWNSGALTSGVHTFPAVLQSSGLYSLSSVVTVPSSSLGTQTYICNVNHKPSNTKVDKKVEPKSCDKTHTCPPCPAPELLGGPSVFLFPPKPKDTLMISRTPEVTCVVVDVSHEDPEVKFNWYVDGVEVHNAKTKPREEQYNSTYRVVSVLTVLHQDWLNGKEYKCKVSNKALPAPIEKTISKAKGQPREPQVYTLPPSREEMTKNQVSLTCLVKGFYPSDIAVEWESNGQPENNYKTTPPVLDSDGSFFLYSKLTVDKSRWQQGNVFSCSVMHEALHNHYTQKSLSLSP

SEQ ID NO: 77 - protein, 444 aa, artificial sequence
QVQLVESGGGVVQPGRSLRLSCVASGFTFSSYGMNWVRQAPGKGLDWVTVIWFDGSNKYYADSVKGRFTISRDNSKNTLYLQMNSLRAEDTAMYYCARGERTLDLWGQGTLVTVSSASTKGPSVFPLAPSSKSTSGGTAALGCLVKDYFPEPVTVSWNSGALTSGVHTFPAVLQSSGLYSLSSVVTVPSSSLGTQTYICNVNHKPSNTKVDKKVEPKSCDKTHTCPPCPAPELLGGPSVFLFPPKPKDTLMISRTPEVTCVVVDVSHEDPEVKFNWYVDGVEVHNAKTKPREEQYNSTYRVVSVLTVLHQDWLNGKEYKCKVSNKALPAPIEKTISKAKGQPREPQVYTLPPSREEMTKNQVSLTCLVKGFYPSDIAVEWESNGQPENNYKTTPPVLDSDGSFFLYSKLTVDKSRWQQGNVFSCSVMHEALHNHYTQKSLSLSP

SEQ ID NO: 78 - protein, 444 aa, artificial sequence
QVQLVESGGGVVQPGRSLRLSCAASGFTFSSYGMNWVRQAPGKGLEWVAVIWFDGSIKYYADSVKGRFTISRDNSKNTLYLQMNSLRAEDTAIYYCARGQLVQDFWGRGTLVTVSSASTKGPSVFPLAPSSKSTSGGTAALGCLVKDYFPEPVTVSWNSGALTSGVHTFPAVLQSSGLYSLSSVVTVPSSSLGTQTYICNVNHKPSNTKVDKKVEPKSCDKTHTCPPCPAPELLGGPSVFLFPPKPKDTLMISRTPEVTCVVVDVSHEDPEVKFNWYVDGVEVHNAKTKPREEQYNSTYRVVSVLTVLHQDWLNGKEYKCKVSNKALPAPIEKTISKAKGQPREPQVYTLPPSREEMTKNQVSLTCLVKGFYPSDIAVEWESNGQPENNYKTTPPVLDSDGSFFLYSKLTVDKSRWQQGNVFSCSVMHEALHNHYTQKSLSLSP

SEQ ID NO: 79 - protein, 444 aa, artificial sequence
QVQLVESGGGVVQPGRSLRLSCAASGFTFSSYGMHWVRQAPGKGLEWVAVIWFDGSLKYYADSVKGRFAISRDNSKNTLYLQMNSLRAEDTAIFYCARGQLVQDLWGRGTLVTVSSASTKGPSVFPLAPSSKSTSGGTAALGCLVKDYFPEPVTVSWNSGALTSGVHTFPAVLQSSGLYSLSSVVTVPSSSLGTQTYICNVNHKPSNTKVDKKVEPKSCDKTHTCPPCPAPELLGGPSVFLFPPKPKDTLMISRTPEVTCVVVDVSHEDPEVKFNWYVDGVEVHNAKTKPREEQYNSTYRVVSVLTVLHQDWLNGKEYKCKVSNKALPAPIEKTISKAKGQPREPQVYTLPPSREEMTKNQVSLTCLVKGFYPSDIAVEWESNGQPENNYKTTPPVLDSDGSFFLYSKLTVDKSRWQQGNVFSCSVMHEALHNHYTQKSLSLSP

SEQ ID NO: 80 - protein, 444 aa, artificial sequence
QVQLVESGGGVVQPGRSLRLSCAASGFTFSSYGMHWVRQAPGKGLEWVAVIWFDGSIKYYADSVKGRFTISRDNSKNTLYLQMNSLRAEDTAIYYCARGQLVQDFWGRGTLVTVSSASTKGPSVFPLAPSSKSTSGGTAALGCLVKDYFPEPVTVSWNSGALTSGVHTFPAVLQSSGLYSLSSVVTVPSSSLGTQTYICNVNHKPSNTKVDKKVEPKSCDKTHTCPPCPAPELLGGPSVFLFPPKPKDTLMISRTPEVTCVVVDVSHEDPEVKFNWYVDGVEVHNAKTKPREEQYNSTYRVVSVLTVLHQDWLNGKEYKCKVSNKALPAPIEKTISKAKGQPREPQVYTLPPSREEMTKNQVSLTCLVKGFYPSDIAVEWESNGQPENNYKTTPPVLDSDGSFFLYSKLTVDKSRWQQGNVFSCSVMHEALHNHYTQKSLSLSP

SEQ ID NO: 81 - protein, 444 aa, artificial sequence
QVQLVESGGGVVQPGRSLRLSCAASGFTFSSYGMHWVRQAPGKGLEWVAVIWFDGSVKYYADSVKGRFTISRDNSKNTLYLQMNSLRAEDTAIYYCARGQLVQDFWGRGTLVTVSSASTKGPSVFPLAPSSKSTSGGTAALGCLVKDYFPEPVTVSWNSGALTSGVHTFPAVLQSSGLYSLSSVVTVPSSSLGTQTYICNVNHKPSNTKVDKKVEPKSCDKTHTCPPCPAPELLGGPSVFLFPPKPKDTLMISRTPEVTCVVVDVSHEDPEVKFNWYVDGVEVHNAKTKPREEQYNSTYRVVSVLTVLHQDWLNGKEYKCKVSNKALPAPIEKTISKAKGQPREPQVYTLPPSREEMTKNQVSLTCLVKGFYPSDIAVEWESNGQPENNYKTTPPVLDSDGSFFLYSKLTVDKSRWQQGNVFSCSVMHEALHNHYTQKSLSLSP

SEQ ID NO: 82 - protein, 446 aa, artificial sequence
EVQLLQSGGGLVQPGGSLRLSCAASGFTFSNYAMTWVRQAPGKGLEWVSTISGSGAFTYYADAVKGRFTISRVNSKNSLDLQMNSLRAEDTAVYYCAKGGILTGFDNWGQGTLVTVSSASTKGPSVFPLAPSSKSTSGGTAALGCLVKDYFPEPVTVSWNSGALTSGVHTFPAVLQSSGLYSLSSVVTVPSSSLGTQTYICNVNHKPSNTKVDKKVEPKSCDKTHTCPPCPAPELLGGPSVFLFPPKPKDTLMISRTPEVTCVVVDVSHEDPEVKFNWYVDGVEVHNAKTKPREEQYNSTYRVVSVLTVLHQDWLNGKEYKCKVSNKALPAPIEKTISKAKGQPREPQVYTLPPSREEMTKNQVSLTCLVKGFYPSDIAVEWESNGQPENNYKTTPPVLDSDGSFFLYSKLTVDKSRWQQGNVFSCSVMHEALHNHYTQKSLSLSP

SEQ ID NO: 83 - protein, 445 aa, artificial sequence
EVQLLESGGGLVQPGGSLRLSCATSGFTFSNYAMTWVRQAPGKGLEWVVISGSGFLTYYADAVKGRFTISRVNSKNSLYLQMNSLRAEDTAVYYCTKGGILTGFDYWGQGTLVTVSSASTKGPSVFPLAPSSKSTSGGTAALGCLVKDYFPEPVTVSWNSGALTSGVHTFPAVLQSSGLYSLSSVVTVPSSSLGTQTYICNVNHKPSNTKVDKKVEPKSCDKTHTCPPCPAPELLGGPSVFLFPPKPKDTLMISRTPEVTCVVVDVSHEDPEVKFNWYVDGVEVHNAKTKPREEQYNSTYRVVSVLTVLHQDWLNGKEYKCKVSNKALPAPIEKTISKAKGQPREPQVYTLPPSREEMTKNQVSLTCLVKGFYPSDIAVEWESNGQPENNYKTTPPVLDSDGSFFLYSKLTVDKSRWQQGNVFSCSVMHEALHNHYTQKSLSLSP

SEQ ID NO: 84 - protein, 215 aa, artificial sequence
EIVLTQSPGTLSLSPGERATLSCRASQSVSSSYLAWYQQKPGQAPRLLIYGASSRATGIPDRFSGSGSGTDFTLTISRLEPEDFAVYYCQQYGSSPFTFGPGTKVDIKRTVAAPSVFIFPPSDEQLKSGTASVVCLLNNFYPREAKVQWKVDNALQSGNSQESVTEQDSKDSTYSLSSTLTLSKADYEKHKVYACEVTHQGLSSPVTKSFNRGEC

SEQ ID NO: 85 - protein, 215 aa, artificial sequence
KIVLTQSPGTLSLSPGGRATLSCRASQSISSSYLAWYQQKPGQAPRLLIYAASNRATGIPDRFSGSGSGTDFTLTISRLEPEDFAVYYCQQYGSSPFTFGPGIKVDIKRTVAAPSVFIFPPSDEQLKSGTASVVCLLNNFYPREAKVQWKVDNALQSGNSQESVTEQDSKDSTYSLSSTLTLSKADYEKHKVYACEVTHQGLSSPVTKSFNRGEC

SEQ ID NO: 86 - protein, 214 aa, artificial sequence
DIQMTQSPSSLSASVGDRVTITCRASQSISSYLNWYQQKPGKAPKLLIYAASSLQSGVPSRFSGSGSGTDFTLTISSLQPEDFATYYCQQSYSTPLTFGGGTKVEIKRTVAAPSVFIFPPSDEQLKSGTASVVCLLNNFYPREAKVQWKVDNALQSGNSQESVTEQDSKDSTYSLSSTLTLSKADYEKHKVYACEVTHQGLSSPVTKSFNRGEC

SEQ ID NO: 87 - protein, 215 aa, artificial sequence
EIVLTQSPGPLSLSPGERATLSCRASQSVSSSFLAWYQQKPGQAPRLLIYGTSSRATGIPDRFSGSGSGTDFTLTISRLEPEDFAVYYCQQYGSSPFTFGPGTKVGIKRTVAAPSVFIFPPSDEQLKSGTASVVCLLNNFYPREAKVQWKVDNALQSGNSQESVTEQDSKDSTYSLSSTLTLSKADYEKHKVYACEVTHQGLSSPVTKSFNRGEC

SEQ ID NO: 88 - protein, 215 aa, artificial sequence
EIVLTQSPGTLSLSPGGRATLSCRASQSVSSSYLAWYQQKPGQAPRLLIYGASSRATGIPDRFSGSGSGTDFTLTISRLEPEDFAVYYCQQYGSSPFTFGPGIKVDIKRTVAAPSVFIFPPSDEQLKSGTASVVCLLNNFYPREAKVQWKVDNALQSGNSQESVTEQDSKDSTYSLSSTLTLSKADYEKHKVYACEVTHQGLSSPVTKSFNRGEC

SEQ ID NO: 89 - protein, 215 aa, artificial sequence; identical to SEQ ID NO: 88

SEQ ID NO: 90 - protein, 217 aa, artificial sequence
DIQMTQSPSTLSASVGDRVTITCRASQSISSWLAWYQQKPGKAPKLLIYKASSLESGVPSRFSGSGSGTEFSFTISSLQPDDFATYYCQQYKSFSPGGLTFGGGTKVEIKRTVAAPSVFIFPPSDEQLKSGTASVVCLLNNFYPREAKVQWKVDNALQSGNSQESVTEQDSKDSTYSLSSTLTLSKADYEKHKVYACEVTHQGLSSPVTKSFNRGEC

SEQ ID NO: 91 - protein, 214 aa, artificial sequence
DIQMTQSPSTLSASVGDRVTITCRASQSISSWLAWYQQKPGKAPNLLMYKASNLESGVPSRFSGSGSGTEFTLTITSLQPDDFASYYCQQYKSNPLTFGGGTKVEIKRTVAAPSVFIFPPSDEQLKSGTASVVCLLNNFYPREAKVQWKVDNALQSGNSQESVTEQDSKDSTYSLSSTLTLSKADYEKHKVYACEVTHQGLSSPVTKSFNRGEC

SEQ ID NO: 92 - protein, 214 aa, artificial sequence
DIQMTQSPSTLSASVGDRVTITCRASQSISSWLAWYQQKPGKAPNLLMYKASNLENGVSSRFSGSGSGTEFTLTITSLQPDDFATYYCQQYKSNPLTFGGGTKVEIKRTVAAPSVFIFPPSDEQLKSGTASVVCLLNNFYPREAKVQWKVDNALQSGNSQESVTEQDSKDSTYSLSSTLTLSKADYEKHKVYACEVTHQGLSSPVTKSFNRGEC

SEQ ID NO: 93 - protein, 214 aa, artificial sequence
KIVMTQSPATLSVSPGERATLSCRASQNLNSNLAWYQQTPGQAPRLLIYGASTRAPGIPARFSGSGSGTEFTLTISSLQSEDFVVYFCQQYNNWPRTFGQGTKVEIKRTVAAPSVFIFPPSDEQLKSGTASVVCLLNNFYPREAKVQWKVDNALQSGNSQESVTEQDSKDSTYSLSSTLTLSKADYEKHKVYACEVTHQGLSSPVTKSFNRGEC

SEQ ID NO: 94 - DNA, 375 bp, artificial sequence
caggtgcagctggtggagtctgggggaggcgtggtccagcctgggaggtccctgagactctcctgtgcagcgtctggattcaccttcagtagctatggcatgcactgggtccgccaggctccaggcaaggggctggagtgggtggcagttatatggtatgatggaaataataaatactatgcggactccgtgaagggccgattcaccatctccagagacaattccaagaacacgctgtatctgcaaatgaatagcctgagagccgaggacacggctgtgtattactgtgcgagagatggggaaagtagtatggttcggggacttcttaactggttcgacccctggggccagggaaccctggtcaccgtctcctca

SEQ ID NO: 95 - DNA, 324 bp, artificial sequence
gaaattgtgttgacgcagtctccaggcaccctgtctttgtctccaggggaaagagccaccctctcctgcagggccagtcagagtgttagcagcagctacttagcctggtaccagcagaaacctggccaggctcccaggctcctcatctatggtgcatccagcagggccactggcatcccagacaggttcagtggcagtgggtctgggacagacttcactctcaccatcagcagactggagcctgaagattttgcagtgtattactgtcagcagtatggtagctcaccattcactttcggccctgggaccaaagtggatatcaaa

SEQ ID NO: 96 - DNA, 354 bp, artificial sequence
gaggtgcaactgttacagtctgggggaggcttggttcagcctggggggtccctgagactctcctgtgcagcctctggattcacctttagtaattatgccatgacctgggtccgccaggctccagggaaggggctggagtgggtctcaactattagtggtagtggtgctttcacatactacgcagacgccgtgaagggccggttcaccatctccagagtcaattccaagaattcgctggatctgcaaatgaacagcctgagagccgaggacacggccgtatattactgtgcgaaaggaggaattcttactgggtttgacaactggggccagggaaccctggtcaccgtctcctca

SEQ ID NO: 97 - DNA, 321 bp, artificial sequence
aaaatagtgatgacgcagtctccagccaccctgtctgtgtctccaggggaaagagccaccctctcctgcagggccagtcagaatcttaacagcaacttagcctggtaccagcagactcctggccaggctcccaggctcctcatctatggtgcatccaccagggcccctggtattccagccaggttcagtggcagtgggtctgggacagagttcactctcaccatcagcagcctgcagtctgaagattttgttgtttatttctgtcagcagtataataactggcctcggacgttcggccaagggaccaaggtggaaatcaaa

SEQ ID NO: 98 - DNA, 366 bp, artificial sequence
caggtgcagctggtggagtctgggggaggcgtggtccagcctgggaggtccctgagactctcctgtgcagcgtctggattcacctttagtagttatggcatggactgggtccgccaggctccaggcaaggggctggagtgggtggcagttatatggtatgatggaagtaataaatactatgcagactccgtgaagggccgattcaccatctccagagacaattccaagaacacgctgtatctgcaaatgaacagcctgagagccgaggacacggctgtttattactgtgcgagagaactatggttcggggagttattatccccttttgacttctggggccagggaaccctggtcaccgtctcctca

SEQ ID NO: 99 - DNA, 324 bp, artificial sequence
aaaattgtgttgacgcagtctccaggcaccctgtctttgtctccagggggaagagccaccctctcctgcagggccagtcagagtattagcagcagctacttagcctggtaccagcagaaacctggccaggctcccaggctcctcatctatgctgcatccaacagggccactggcatcccagacaggttcagtggcagtgggtctgggacagacttcactctcaccatcagcagactggagcctgaagattttgcagtgtattactgtcagcagtatggtagctcaccattcactttcggccctgggatcaaagtggatatcaaa

SEQ ID NO: 100 - DNA, 366 bp, artificial sequence
caggtgcagctggtggagtctgggggaggcgtggtccagcctgggaggtccctgagactctcctgtgcagcgtctggattcacctttagtagttatggcatggactgggtccgccaggctccaggcaaggggctggagtgggtggcagttatatggtatgatggaagtaataaattctatgcagactccgtgaggggccgattcaccatctccagagacaattcccagaacacgctgtatctgcaaatgaacagcctgagagccgaggacacggctgtttattactgtgcgagagaactctggttcggggagttattatcccctcttgacttctggggccagggaaccctggtcaccgtctcctca

SEQ ID NO: 101 - DNA, 324 bp, artificial sequence
gaaattgtgttgacgcagtctccaggcaccctgtctttgtctccagggggaagagccaccctctcctgcagggccagtcagagtgttagcagcagctacttagcctggtaccagcagaaacctggccaggctcccaggctcctcatctatggtgcatccagcagggccactggcatcccagacaggttcagtggcagtgggtctgggacagacttcactctcaccatcagcagactggagcctgaagattttgcagtgtattactgtcagcagtatggtagctcaccattcactttcggccctgggatcaaagtggatatcaaa

SEQ ID NO: 102 - DNA, 348 bp, artificial sequence
caggtgcagctggtggagtctgggggaggcgtggtccagcctgggaggtccctgagactctcctgtgcagcgtctggattcaccttcagtagctatggcatgcactgggtccgccaggctccaggcaagggactggagtgggtggcagttatatggtttgatggaagtcttaaatactatgcagactccgtgaagggccgattcgccatctccagagacaattccaagaacacgctctatctgcaaatgaacagcctgagagccgaggacacggctatattttactgtgcgcgagggcagctggtgcaggacctctggggccggggaaccctggtcaccgtctcctca

SEQ ID NO: 103 - DNA, 321 bp, artificial sequence
gacatccagatgacccagtctccttccaccctgtctgcatctgtaggagacagagtcaccatcacttgccgggccagtcagagtattagtagctggttggcctggtatcagcagaaaccagggaaagcccctaacctcctgatgtataaggcgtctaatttagaaagtggggtcccatcaaggttcagcggcagtggatctgggacagaattcactctcaccatcaccagcctgcagcctgatgattttgcaagttattactgccaacagtataaaagtaatccgctcactttcggcggagggaccaaggtggagatcaaa